European Patent Application EP 4 385 458 A1, published June 19, 2024. Title: Oral film with multiple regions for therapy of periodontal and dental diseases or disorders. Applicant: vVardis AG. Application EP. The sequence listing filed with the application follows.

SEQUENCE LISTING (33 sequences)

SEQ ID NO: 1-4 - skipped (4 entries)

SEQ ID NO: 5 - protein, 11 aa, synthetic construct
  REGION 1..11: note = consensus sequence 5 of self-assembling peptides
  VARIANT 5: note = amino acid X1 is independently selected from the group consisting of glutamic acid and ornithine
  VARIANT 7: note = amino acid X1 is independently selected from the group consisting of glutamic acid and ornithine
  VARIANT 9: note = amino acid X1 is independently selected from the group consisting of glutamic acid and ornithine
QQRFXWXFXQQ

SEQ ID NO: 6 - protein, 11 aa, synthetic construct
  REGION 1..11: note = P11-4
QQRFEWEFEQQ

SEQ ID NO: 7 - protein, 11 aa, synthetic construct
  REGION 1..11: note = P11-2
QQRFQWQFEQQ

SEQ ID NO: 8 - protein, 11 aa, synthetic construct
  REGION 1..11: note = P11-5
  MOD_RES 5: note = ornithine
  MOD_RES 7: note = ornithine
QQRFXWXFQQQ

SEQ ID NO: 9 - protein, 11 aa, synthetic construct
  REGION 1..11: note = P11-8
  MOD_RES 5: note = ornithine
  MOD_RES 7: note = ornithine
QQRFXWXFEQQ

SEQ ID NO: 10 - protein, 11 aa, synthetic construct
  REGION 1..11: note = P11-12
  MOD_RES 5: note = ornithine
  MOD_RES 7: note = ornithine
SSRFXWXFESS

SEQ ID NO: 11 - protein, 11 aa, synthetic construct
  REGION 1..11: note = P11-13
EQEFEWEFEQE

SEQ ID NO: 12 - protein, 11 aa, synthetic construct
  REGION 1..11: note = P11-14
  MOD_RES 3: note = ornithine
  MOD_RES 5: note = ornithine
  MOD_RES 7: note = ornithine
  MOD_RES 9: note = ornithine
QQXFXWXFXQQ

SEQ ID NO: 13 - protein, 11 aa, synthetic construct
  REGION 1..11: note = P11-17
TTRFEWEFETT

SEQ ID NO: 14 - protein, 11 aa, synthetic construct
  REGION 1..11: note = P11-19
  MOD_RES 5: note = ornithine
  MOD_RES 7: note = ornithine
QQRQXQXQEQQ

SEQ ID NO: 15 - protein, 11 aa, synthetic construct
  REGION 1..11: note = P11-20
QQRQEQEQEQQ

SEQ ID NO: 16 - protein, 11 aa, synthetic construct
  MOD_RES 1: note = ornithine
  REGION 1..11: note = P11-28
  MOD_RES 3: note = ornithine
  MOD_RES 5: note = ornithine
  MOD_RES 7: note = ornithine
  MOD_RES 9: note = ornithine
  MOD_RES 11: note = ornithine
XQXFXWXFXQX

SEQ ID NO: 17 - protein, 11 aa, synthetic construct
  REGION 1..11: note = P11-29
QQEFEWEFEQQ

SEQ ID NO: 18 - protein, 11 aa, synthetic construct
  MOD_RES 1: note = ACETYLATION
  REGION 1..11: note = P11-4mod
  MOD_RES 11: note = AMIDATION
QQRFEWEFEQQ

SEQ ID NO: 19 - protein, 11 aa, synthetic construct
  MOD_RES 1: note = ACETYLATION
  REGION 1..11: note = P11-2mod
  MOD_RES 11: note = AMIDATION
QQRFQWQFEQQ

SEQ ID NO: 20 - protein, 11 aa, synthetic construct
  MOD_RES 1: note = ACETYLATION
  REGION 1..11: note = P11-5mod
  MOD_RES 5: note = ornithine
  MOD_RES 7: note = ornithine
  MOD_RES 11: note = AMIDATION
QQRFXWXFQQQ

SEQ ID NO: 21 - protein, 11 aa, synthetic construct
  MOD_RES 1: note = ACETYLATION
  REGION 1..11: note = P11-8mod
  MOD_RES 5: note = ornithine
  MOD_RES 7: note = ornithine
  MOD_RES 11: note = AMIDATION
QQRFXWXFEQQ

SEQ ID NO: 22 - protein, 11 aa, synthetic construct
  MOD_RES 1: note = ACETYLATION
  REGION 1..11: note = P11-12mod
  MOD_RES 5: note = ornithine
  MOD_RES 7: note = ornithine
  MOD_RES 11: note = AMIDATION
SSRFXWXFESS

SEQ ID NO: 23 - protein, 11 aa, synthetic construct
  MOD_RES 1: note = ACETYLATION
  REGION 1..11: note = P11-13mod
  MOD_RES 11: note = AMIDATION
EQEFEWEFEQE

SEQ ID NO: 24 - protein, 11 aa, synthetic construct
  MOD_RES 1: note = ACETYLATION
  REGION 1..11: note = P11-14mod
  MOD_RES 3: note = ornithine
  MOD_RES 5: note = ornithine
  MOD_RES 7: note = ornithine
  MOD_RES 9: note = ornithine
  MOD_RES 11: note = AMIDATION
QQXFXWXFXQQ

SEQ ID NO: 25 - protein, 11 aa, synthetic construct
  MOD_RES 1: note = ACETYLATION
  REGION 1..11: note = P11-17mod
  MOD_RES 11: note = AMIDATION
TTRFEWEFETT

SEQ ID NO: 26 - protein, 11 aa, synthetic construct
  MOD_RES 1: note = ACETYLATION
  REGION 1..11: note = P11-19mod
  MOD_RES 5: note = ornithine
  MOD_RES 7: note = ornithine
  MOD_RES 11: note = AMIDATION
QQRQXQXQEQQ

SEQ ID NO: 27 - protein, 11 aa, synthetic construct
  MOD_RES 1: note = ACETYLATION
  REGION 1..11: note = P11-20mod
  MOD_RES 11: note = AMIDATION
QQRQEQEQEQQ

SEQ ID NO: 28 - protein, 11 aa, synthetic construct
  MOD_RES 1: note = ACETYLATION
  MOD_RES 1: note = ornithine
  REGION 1..11: note = P11-28mod
  MOD_RES 3: note = ornithine
  MOD_RES 5: note = ornithine
  MOD_RES 7: note = ornithine
  MOD_RES 9: note = ornithine
  MOD_RES 11: note = ornithine
  MOD_RES 11: note = AMIDATION
XQXFXWXFXQX

SEQ ID NO: 29 - protein, 11 aa, synthetic construct
  MOD_RES 1: note = ACETYLATION
  REGION 1..11: note = P11-29mod
  MOD_RES 11: note = AMIDATION
QQEFEWEFEQQ

SEQ ID NO: 30 - protein, 11 aa, synthetic construct
  REGION 1..11: note = P11-16
  MOD_RES 5: note = ornithine
  MOD_RES 7: note = ornithine
NNRFXWXFENN

SEQ ID NO: 31 - protein, 11 aa, synthetic construct
  REGION 1..11: note = P11-18
  MOD_RES 5: note = ornithine
  MOD_RES 7: note = ornithine
TTRFXWXFETT

SEQ ID NO: 32 - protein, 11 aa, synthetic construct
  REGION 1..11: note = P11-26
  MOD_RES 3: note = ornithine
  MOD_RES 5: note = ornithine
  MOD_RES 7: note = ornithine
  MOD_RES 9: note = ornithine
QQXQXQXQXQQ

SEQ ID NO: 33 - protein, 11 aa, synthetic construct
  REGION 1..11: note = P11-31
  MOD_RES 3: note = ornithine
  MOD_RES 5: note = ornithine
  MOD_RES 7: note = ornithine
  MOD_RES 9: note = ornithine
SSXFXWXFXSS